European Patent Application EP 4 292 607 A1, published December 20, 2023. Title: STABLE PREPARATION OF HUMAN PAPILLOMAVIRUS VIRUS-LIKE PARTICLE VACCINE. Applicant: SINOCELLTECH LTD. Application EP22739080.4. The sequence listing filed with the application follows.

SEQUENCE LISTING (41 sequences)

SEQ ID NO: 1 - protein, 26 aa, Artificial
  The sequence is artificially synthesized.
KAKPKLKRAAPTSTRTSSAKRKKVKK

SEQ ID NO: 2 - protein, 31 aa, Artificial
  The sequence is artificially synthesized.
LQAGLKAKPKLKRAAPTSTRTSSAKRKKVKK

SEQ ID NO: 3 - protein, 38 aa, Artificial
  The sequence is artificially synthesized.
LQLGARPKPTIGPRKRAAPAPTSTPSPKRVKRRKSSRK

SEQ ID NO: 4 - protein, 469 aa, Artificial
  The sequence is artificially synthesized.
MWRPSDSTVYVPPPNPVSKVVATDAYVTRTNIFYHASSSRLLAVGHPYFSIKRANKTVVPKVSGYQYRVFKVVLPDPNKFALPDSSLFDPTTQRLVWACTGLEVGRGQPLGVGVSGHPFLNKYDDVENSGSGGNPGQDNRVNVGMDYKQTQLCMVGCAPPLGEHWGKGKQCTNTPVQAGDCPPLELITSVIQDGDMVDTGFGAMNFADLQTNKSDVPIDICGTTCKYPDYLQMAADPYGDRLFFFLRKEQMFARHFFNRAGEVGEPVPDTLIIKGSGNRTSVGSSIYVNTPSGSLVSSEAQLFNKPYWLQKAQGHNNGICWGNQLFVTVVDTTRSTNMTLCASVTTSSTYTNSDYKEYMRHVEEYDLQFIFQLCSITLSAEVMAYIHTMNPSVLEDWNFGLSPPPNGTLEDTYRYVQSQAITCQKPTPEKEKPDPYKNLSFWEVNLKEKFSSELDQYPLGRKFLLQSGY

SEQ ID NO: 5 - protein, 470 aa, Artificial
  The sequence is artificially synthesized.
MWRPSDSTVYVPPPNPVSKVVATDAYVKRTNIFYHASSSRLLAVGHPYYSIKKVNKTVVPKVSGYQYRVFKVVLPDPNKFALPDSSLFDPTTQRLVWACTGLEVGRGQPLGVGVSGHPLLNKYDDVENSGGYGGNPGQDNRVNVGMDYKQTQLCMVGCAPPLGEHWGKGTQCSNTSVQNGDCPPLELITSVIQDGDMVDTGFGAMNFADLQTNKSDVPLDICGTVCKYPDYLQMAADPYGDRLFFYLRKEQMFARHFFNRAGTVGEPVPDDLLVKGGNNRSSVASSIYVHTPSGSLVSSEAQLFNKPYWLQKAQGHNNGICWGNHLFVTVVDTTRSTNMTLCASVSKSATYTNSDYKEYMRHVEEFDLQFIFQLCSITLSAEVMAYIHTMNPSVLEDWNFGLSPPPNGTLEDTYRYVQSQAITCQKPTPEKEKQDPYKDMSFWEVNLKEKFSSELDQFPLGRKFLLQSGY

SEQ ID NO: 6 - protein, 474 aa, Artificial
  The sequence is artificially synthesized.
MSLWLPSEATVYLPPVPVSKVVSTDEYVARTNIYYHAGTSRLLAVGHPYFPIKKPNNNKILVPKVSGLQYRVFRIHLPDPNKFGFPDTSFYNPDTQRLVWACVGVEVGRGQPLGVGISGHPLLNKLDDTENASAYAANAGVDNRECISMDYKQTQLCLIGCKPPIGEHWGKGSPCTNVAVNPGDCPPLELINTVIQDGDMVDTGFGAMDFTTLQANKSEVPLDICTSICKYPDYIKMVSEPYGDSLFFYLRREQMFVRHLFNRAGAVGENVPDDLYIKGSGSTANLASSNYFPTPSGSMVTSDAQIFNKPYWLQRAQGHNNGICWGNQLFVTVVDTTRSTNMSLCAAISTSETTYKNTNFKEYLRHGEEYDLQFIFQLCKITLTADVMTYIHSMNSTILEDWNFGLQPPPGGTLEDTYRFVTSQAIACQKHTPPAPKEDPLKKYTFWEVNLKEKFSADLDQFPLGRKFLLQAGL

SEQ ID NO: 7 - protein, 470 aa, Artificial
  The sequence is artificially synthesized.
MALWRPSDNTVYLPPPSVARVVNTDDYVTRTSIFYHAGSSRLLTVGNPYFRVPAGGGNKQDIPKVSAYQYRVFRVQLPDPNKFGLPDTSIYNPETQRLVWACAGVEIGRGQPLGVGLSGHPFYNKLDDTESSHAATSNVSEDVRDNVSVDYKQTQLCILGCAPAIGEHWAKGTACKSRPLSQGDCPPLELKNTVLEDGDMVDTGYGAMDFSTLQDTKCEVPLDICQSICKYPDYLQMSADPYGDSMFFCLRREQLFARHFWNRAGTMGDTVPQSLYIKGTGMRASPGSCVYSPSPSGSIVTSDSQLFNKPYWLHKAQGHNNGVCWHNQLFVTVVDTTRSTNLTICASTQSPVPGQYDATKFKQYSRHVEEYDLQFIFQLCTITLTADVMSYIHSMNSSILEDWNFGVPPPPTTSLVDTYRFVQSVAITCQKDAAPAENKDPYDKLKFWNVDLKEKFSLDLDQYPLGRKFL

SEQ ID NO: 8 - protein, 475 aa, Artificial
  The sequence is artificially synthesized.
MSLWRPSEATVYLPPVPVSKVVSTDEYVTRTNIYYHAGSARLLTVGHPYYSIPKSDNPKKIVVPKVSGLQYRVFRVRLPDPNKFGFPDTSFYNPETQRLVWACVGLEVGRGQPLGVGISGHPLLNKFDDTENSNRYAGGPGTDNRECISMDYKQTQLCLLGCKPPIGEHWGKGSPCSNNAITPGDCPPLELKNSVIQDGDMVDTGFGAMDFTALQDTKSNVPLDICNSICKYPDYLKMVAEPYGDTLFFYLRREQMFVRHFFNRSGTVGESVPTDLYIKGSGSTATLANSTYFPTPSGSMVTSDAQIFNKPYWMQRAQGHNNGICWGNQLFVTVVDTTRSTNMSVCAAIANSDTTFKSSNFKEYLRHGEEFDLQFIFQLCKITLSADIMTYIHSMNPAILEDWNFGLTTPPSGSLEDTYRFVTSQAITCQKSAPQKPKEDPFKDYVFWEVNLKEKFSADLDQFPLGRKFLLQAGY

SEQ ID NO: 9 - protein, 472 aa, Artificial
  The sequence is artificially synthesized.
MSLWRSNEATVYLPPVSVSKVVSTDEYVTRTNIYYHAGSSRLLAVGHPYYAIKKQDSNKIAVPKVSGLQYRVFRVKLPDPNKFGFPDTSFYDPASQRLVWACTGVEVGRGQPLGVGISGHPLLNKLDDTENSNKYVGNSGTDNRECISMDYKQTQLCLIGCRPPIGEHWGKGTPCNANQVKAGECPPLELLNTVLQDGDMVDTGFGAMDFTTLQANKSDVPLDICSSICKYPDYLKMVSEPYGDMLFFYLRREQMFVRHLFNRAGTVGETVPADLYIKGTTGTLPSTSYFPTPSGSMVTSDAQIFNKPYWLQRAQGHNNGICWSNQLFVTVVDTTRSTNMSVCSAVSSSDSTYKNDNFKEYLRHGEEYDLQFIFQLCKITLTADVMTYIHSMNPSILEDWNFGLTPPPSGTLEDTYRYVTSQAVTCQKPSAPKPKDDPLKNYTFWEVDLKEKFSADLDQFPLGRKFLLQAGL

SEQ ID NO: 10 - protein, 469 aa, Artificial
  The sequence is artificially synthesized.
MAMWRSSDSMVYLPPPSVAKVVNTDDYVTRTGIYYYAGSSRLLTVGHPYFKVGMNGGRKQDIPKVSAYQYRVFRVTLPDPNKFSIPDASLYNPETQRLVWACVGVEVGRGQPLGVGISGHPLYNRQDDTENSPFSSTTNKDSRDNVSVDYKQTQLCIIGCVPAIGEHWGKGKACKPNNVSTGDCPPLELVNTPIEDGDMIDTGYGAMDFGALQETKSEVPLDICQSICKYPDYLQMSADVYGDSMFFCLRREQLFARHFWNRGGMVGDAIPAQLYIKGTDIRANPGSSVYCPSPSGSMVTSDSQLFNKPYWLHKAQGHNNGICWHNQLFLTVVDTTRSTNFTLSTSIESSIPSTYDPSKFKEYTRHVEEYDLQFIFQLCTVTLTTDVMSYIHTMNSSILDNWNFAVAPPPSASLVDTYRYLQSAAITCQKDAPAPEKKDPYDGLKFWNVDLREKFSLELDQFPLGRKFL

SEQ ID NO: 11 - protein, 478 aa, Artificial
  The sequence is artificially synthesized.
MALWRPSDSTVYLPPPSVARVVNTDDYVSRTSIFYHAGSSRLLTVGNPYFRVVPSGAGNKQAVPKVSAYQYRVFRVALPDPNKFGLPDSTIYNPETQRLVWACVGMEIGRGQPLGIGLSGHPFYNKLDDTESAHAATAVITQDVRDNVSVDYKQTQLCILGCVPAIGEHWAKGTLCKPAQLQPGDCPPLELKNTIIEDGDMVDTGYGAMDFSTLQDTKCEVPLDICQSICKYPDYLQMSADPYGDSMFFCLRREQLFARHFWNRAGVMGDTVPTDLYIKGTSANMRETPGSCVYSPSPSGSITTSDSQLFNKPYWLHKAQGHNNGICWHNQLFVTVVDTTRSTNLTLCASTQNPVPNTYDPTKFKHYSRHVEEYDLQFIFQLCTITLTAEVMSYIHSMNSSILENWNFGVPPPPTTSLVDTYRFVQSVAVTCQKDTTPPEKQDPYDKLKFWTVDLKEKFSSDLDQYPLGRKFLVQAGL

SEQ ID NO: 12 - protein, 474 aa, Artificial
  The sequence is artificially synthesized.
MALWRTNDSKVYLPPAPVSRIVNTEEYITRTGIYYYAGSSRLITLGHPYFPIPKTSTRAAIPKVSAFQYRVFRVQLPDPNKFGLPDPNLYNPDTDRLVWGCVGVEVGRGQPLGVGLSGHPLFNKYDDTENSRIANGNAQQDVRDNTSVDNKQTQLCIIGCAPPIGEHWGIGTTCKNTPVPPGDCPPLELVSSVIQDGDMIDTGFGAMDFAALQATKSDVPLDISQSVCKYPDYLKMSADTYGNSMFFHLRREQIFARHYYNKLVGVGEDIPNDYYIKGSGNGRDPIESYIYSATPSGSMITSDSQIFNKPYWLHRAQGHNNGICWNNQLFITCVDTTRSTNLTISTATAAVSPTFTPSNFKQYIRHGEEYELQFIFQLCKITLTTEVMAYLHTMDPTILEQWNFGLTLPPSASLEDAYRFVRNAATSCQKDTPPQAKPDPLAKYKFWDVDLKERFSLDLDQFALGRKFLLQVGV

SEQ ID NO: 13 - protein, 478 aa, Artificial
  The sequence is artificially synthesized.
MSVWRPSEATVYLPPVPVSKVVSTDEYVSRTSIYYYAGSSRLLTVGHPYFSIKNTSSGNGKKVLVPKVSGLQYRVFRIKLPDPNKFGFPDTSFYNPETQRLVWACTGLEIGRGQPLGVGISGHPLLNKFDDTETSNKYAGKPGIDNRECLSMDYKQTQLCILGCKPPIGEHWGKGTPCNNNSGNPGDCPPLQLINSVIQDGDMVDTGFGCMDFNTLQASKSDVPIDICSSVCKYPDYLQMASEPYGDSLFFFLRREQMFVRHFFNRAGTLGDPVPGDLYIQGSNSGNTATVQSSAFFPTPSGSMVTSESQLFNKPYWLQRAQGHNNGICWGNQLFVTVVDTTRSTNMTLCAEVKKESTYKNENFKEYLRHGEEFDLQFIFQLCKITLTADVMTYIHKMDATILEDWQFGLTPPPSASLEDTYRFVTSTAITCQKNTPPKGKEDPLKDYMFWEVDLKEKFSADLDQFPLGRKFLLQAGL

SEQ ID NO: 14 - protein, 467 aa, Artificial
  The sequence is artificially synthesized.
MATWRPSENKVYLPPTPVSKVVATDSYVKRTSIFYHAGSSRLLAVGHPYYSVTKDNTKTNIPKVSAYQYRVFRVRLPDPNKFGLPDTNIYNPDQERLVWACVGLEVGRGQPLGAGLSGHPLFNRLDDTESSNLANNNVIEDSRDNISVDGKQTQLCIVGCTPAMGEHWTKGAVCKSTQVTTGDCPPLALINTPIEDGDMIDTGFGAMDFKVLQESKAEVPLDIVQSTCKYPDYLKMSADAYGDSMWFYLRREQLFARHYFNRAGKVGETIPAELYLKGSNGREPPPSSVYVATPSGSMITSEAQLFNKPYWLQRAQGHNNGICWGNQLFVTVVDTTRSTNMTISTATEQLSKYDARKINQYLRHVEEYELQFVFQLCKITLSAEVMAYLHNMNANLLEDWNIGLSPPVATSLEDKYRYVRSTAITCQREQPPTEKQDPLAKYKFWDVNLQDSFSTDLDQFPLGRKFL

SEQ ID NO: 15 - protein, 473 aa, Artificial
  The sequence is artificially synthesized.
MSVWRPSEATVYLPPVPVSKVVSTDEYVSRTSIYYYAGSSRLLAVGNPYFSIKSPNNNKKVLVPKVSGLQYRVFRVRLPDPNKFGFPDTSFYNPDTQRLVWACVGLEIGRGQPLGVGVSGHPYLNKFDDTETSNRYPAQPGSDNRECLSMDYKQTQLCLIGCKPPTGEHWGKGVACNNNAAATDCPPLELFNSIIEDGDMVDTGFGCMDFGTLQANKSDVPIDICNSTCKYPDYLKMASEPYGDSLFFFLRREQMFVRHFFNRAGKLGEAVPDDLYIKGSGNTAVIQSSAFFPTPSGSIVTSESQLFNKPYWLQRAQGHNNGICWGNQLFVTVVDTTRSTNMTLCTEVTKEGTYKNDNFKEYVRHVEEYDLQFVFQLCKITLTAEIMTYIHTMDSNILEDWQFGLTPPPSASLQDTYRFVTSQAITCQKTAPPKEKEDPLNKYTFWEVNLKEKFSADLDQFPLGRKFLLQSGL

SEQ ID NO: 16 - protein, 495 aa, Artificial
  The sequence is artificially synthesized.
MWRPSDSTVYVPPPNPVSKVVATDAYVTRTNIFYHASSSRLLAVGHPYFSIKRANKTVVPKVSGYQYRVFKVVLPDPNKFALPDSSLFDPTTQRLVWACTGLEVGRGQPLGVGVSGHPFLNKYDDVENSGSGGNPGQDNRVNVGMDYKQTQLCMVGCAPPLGEHWGKGKQCTNTPVQAGDCPPLELITSVIQDGDMVDTGFGAMNFADLQTNKSDVPIDICGTTCKYPDYLQMAADPYGDRLFFFLRKEQMFARHFFNRAGEVGEPVPDTLIIKGSGNRTSVGSSIYVNTPSGSLVSSEAQLFNKPYWLQKAQGHNNGICWGNQLFVTVVDTTRSTNMTLCASVTTSSTYTNSDYKEYMRHVEEYDLQFIFQLCSITLSAEVMAYIHTMNPSVLEDWNFGLSPPPNGTLEDTYRYVQSQAITCQKPTPEKEKPDPYKNLSFWEVNLKEKFSSELDQYPLGRKFLLQSGYKAKPKLKRAAPTSTRTSSAKRKKVKK

SEQ ID NO: 17 - protein, 496 aa, Artificial
  The sequence is artificially synthesized.
MWRPSDSTVYVPPPNPVSKVVATDAYVKRTNIFYHASSSRLLAVGHPYYSIKKVNKTVVPKVSGYQYRVFKVVLPDPNKFALPDSSLFDPTTQRLVWACTGLEVGRGQPLGVGVSGHPLLNKYDDVENSGGYGGNPGQDNRVNVGMDYKQTQLCMVGCAPPLGEHWGKGTQCSNTSVQNGDCPPLELITSVIQDGDMVDTGFGAMNFADLQTNKSDVPLDICGTVCKYPDYLQMAADPYGDRLFFYLRKEQMFARHFFNRAGTVGEPVPDDLLVKGGNNRSSVASSIYVHTPSGSLVSSEAQLFNKPYWLQKAQGHNNGICWGNHLFVTVVDTTRSTNMTLCASVSKSATYTNSDYKEYMRHVEEFDLQFIFQLCSITLSAEVMAYIHTMNPSVLEDWNFGLSPPPNGTLEDTYRYVQSQAITCQKPTPEKEKQDPYKDMSFWEVNLKEKFSSELDQFPLGRKFLLQSGYKAKPKLKRAAPTSTRTSSAKRKKVKK

SEQ ID NO: 18 - protein, 500 aa, Artificial
  The sequence is artificially synthesized.
MSLWLPSEATVYLPPVPVSKVVSTDEYVARTNIYYHAGTSRLLAVGHPYFPIKKPNNNKILVPKVSGLQYRVFRIHLPDPNKFGFPDTSFYNPDTQRLVWACVGVEVGRGQPLGVGISGHPLLNKLDDTENASAYAANAGVDNRECISMDYKQTQLCLIGCKPPIGEHWGKGSPCTNVAVNPGDCPPLELINTVIQDGDMVDTGFGAMDFTTLQANKSEVPLDICTSICKYPDYIKMVSEPYGDSLFFYLRREQMFVRHLFNRAGAVGENVPDDLYIKGSGSTANLASSNYFPTPSGSMVTSDAQIFNKPYWLQRAQGHNNGICWGNQLFVTVVDTTRSTNMSLCAAISTSETTYKNTNFKEYLRHGEEYDLQFIFQLCKITLTADVMTYIHSMNSTILEDWNFGLQPPPGGTLEDTYRFVTSQAIACQKHTPPAPKEDPLKKYTFWEVNLKEKFSADLDQFPLGRKFLLQAGLKAKPKLKRAAPTSTRTSSAKRKKVKK

SEQ ID NO: 19 - protein, 496 aa, Artificial
  The sequence is artificially synthesized.
MALWRPSDNTVYLPPPSVARVVNTDDYVTRTSIFYHAGSSRLLTVGNPYFRVPAGGGNKQDIPKVSAYQYRVFRVQLPDPNKFGLPDTSIYNPETQRLVWACAGVEIGRGQPLGVGLSGHPFYNKLDDTESSHAATSNVSEDVRDNVSVDYKQTQLCILGCAPAIGEHWAKGTACKSRPLSQGDCPPLELKNTVLEDGDMVDTGYGAMDFSTLQDTKCEVPLDICQSICKYPDYLQMSADPYGDSMFFCLRREQLFARHFWNRAGTMGDTVPQSLYIKGTGMRASPGSCVYSPSPSGSIVTSDSQLFNKPYWLHKAQGHNNGVCWHNQLFVTVVDTTRSTNLTICASTQSPVPGQYDATKFKQYSRHVEEYDLQFIFQLCTITLTADVMSYIHSMNSSILEDWNFGVPPPPTTSLVDTYRFVQSVAITCQKDAAPAENKDPYDKLKFWNVDLKEKFSLDLDQYPLGRKFLKAKPKLKRAAPTSTRTSSAKRKKVKK

SEQ ID NO: 20 - protein, 501 aa, Artificial
  The sequence is artificially synthesized.
MSLWRPSEATVYLPPVPVSKVVSTDEYVTRTNIYYHAGSARLLTVGHPYYSIPKSDNPKKIVVPKVSGLQYRVFRVRLPDPNKFGFPDTSFYNPETQRLVWACVGLEVGRGQPLGVGISGHPLLNKFDDTENSNRYAGGPGTDNRECISMDYKQTQLCLLGCKPPIGEHWGKGSPCSNNAITPGDCPPLELKNSVIQDGDMVDTGFGAMDFTALQDTKSNVPLDICNSICKYPDYLKMVAEPYGDTLFFYLRREQMFVRHFFNRSGTVGESVPTDLYIKGSGSTATLANSTYFPTPSGSMVTSDAQIFNKPYWMQRAQGHNNGICWGNQLFVTVVDTTRSTNMSVCAAIANSDTTFKSSNFKEYLRHGEEFDLQFIFQLCKITLSADIMTYIHSMNPAILEDWNFGLTTPPSGSLEDTYRFVTSQAITCQKSAPQKPKEDPFKDYVFWEVNLKEKFSADLDQFPLGRKFLLQAGYKAKPKLKRAAPTSTRTSSAKRKKVKK

SEQ ID NO: 21 - protein, 498 aa, Artificial
  The sequence is artificially synthesized.
MSLWRSNEATVYLPPVSVSKVVSTDEYVTRTNIYYHAGSSRLLAVGHPYYAIKKQDSNKIAVPKVSGLQYRVFRVKLPDPNKFGFPDTSFYDPASQRLVWACTGVEVGRGQPLGVGISGHPLLNKLDDTENSNKYVGNSGTDNRECISMDYKQTQLCLIGCRPPIGEHWGKGTPCNANQVKAGECPPLELLNTVLQDGDMVDTGFGAMDFTTLQANKSDVPLDICSSICKYPDYLKMVSEPYGDMLFFYLRREQMFVRHLFNRAGTVGETVPADLYIKGTTGTLPSTSYFPTPSGSMVTSDAQIFNKPYWLQRAQGHNNGICWSNQLFVTVVDTTRSTNMSVCSAVSSSDSTYKNDNFKEYLRHGEEYDLQFIFQLCKITLTADVMTYIHSMNPSILEDWNFGLTPPPSGTLEDTYRYVTSQAVTCQKPSAPKPKDDPLKNYTFWEVDLKEKFSADLDQFPLGRKFLLQAGLKAKPKLKRAAPTSTRTSSAKRKKVKK

SEQ ID NO: 22 - protein, 507 aa, Artificial
  The sequence is artificially synthesized.
MAMWRSSDSMVYLPPPSVAKVVNTDDYVTRTGIYYYAGSSRLLTVGHPYFKVGMNGGRKQDIPKVSAYQYRVFRVTLPDPNKFSIPDASLYNPETQRLVWACVGVEVGRGQPLGVGISGHPLYNRQDDTENSPFSSTTNKDSRDNVSVDYKQTQLCIIGCVPAIGEHWGKGKACKPNNVSTGDCPPLELVNTPIEDGDMIDTGYGAMDFGALQETKSEVPLDICQSICKYPDYLQMSADVYGDSMFFCLRREQLFARHFWNRGGMVGDAIPAQLYIKGTDIRANPGSSVYCPSPSGSMVTSDSQLFNKPYWLHKAQGHNNGICWHNQLFLTVVDTTRSTNFTLSTSIESSIPSTYDPSKFKEYTRHVEEYDLQFIFQLCTVTLTTDVMSYIHTMNSSILDNWNFAVAPPPSASLVDTYRYLQSAAITCQKDAPAPEKKDPYDGLKFWNVDLREKFSLELDQFPLGRKFLLQLGARPKPTIGPRKRAAPAPTSTPSPKRVKRRKSSRK

SEQ ID NO: 23 - protein, 504 aa, Artificial
  The sequence is artificially synthesized.
MALWRPSDSTVYLPPPSVARVVNTDDYVSRTSIFYHAGSSRLLTVGNPYFRVVPSGAGNKQAVPKVSAYQYRVFRVALPDPNKFGLPDSTIYNPETQRLVWACVGMEIGRGQPLGIGLSGHPFYNKLDDTESAHAATAVITQDVRDNVSVDYKQTQLCILGCVPAIGEHWAKGTLCKPAQLQPGDCPPLELKNTIIEDGDMVDTGYGAMDFSTLQDTKCEVPLDICQSICKYPDYLQMSADPYGDSMFFCLRREQLFARHFWNRAGVMGDTVPTDLYIKGTSANMRETPGSCVYSPSPSGSITTSDSQLFNKPYWLHKAQGHNNGICWHNQLFVTVVDTTRSTNLTLCASTQNPVPNTYDPTKFKHYSRHVEEYDLQFIFQLCTITLTAEVMSYIHSMNSSILENWNFGVPPPPTTSLVDTYRFVQSVAVTCQKDTTPPEKQDPYDKLKFWTVDLKEKFSSDLDQYPLGRKFLVQAGLKAKPKLKRAAPTSTRTSSAKRKKVKK

SEQ ID NO: 24 - protein, 500 aa, Artificial
  The sequence is artificially synthesized.
MALWRTNDSKVYLPPAPVSRIVNTEEYITRTGIYYYAGSSRLITLGHPYFPIPKTSTRAAIPKVSAFQYRVFRVQLPDPNKFGLPDPNLYNPDTDRLVWGCVGVEVGRGQPLGVGLSGHPLFNKYDDTENSRIANGNAQQDVRDNTSVDNKQTQLCIIGCAPPIGEHWGIGTTCKNTPVPPGDCPPLELVSSVIQDGDMIDTGFGAMDFAALQATKSDVPLDISQSVCKYPDYLKMSADTYGNSMFFHLRREQIFARHYYNKLVGVGEDIPNDYYIKGSGNGRDPIESYIYSATPSGSMITSDSQIFNKPYWLHRAQGHNNGICWNNQLFITCVDTTRSTNLTISTATAAVSPTFTPSNFKQYIRHGEEYELQFIFQLCKITLTTEVMAYLHTMDPTILEQWNFGLTLPPSASLEDAYRFVRNAATSCQKDTPPQAKPDPLAKYKFWDVDLKERFSLDLDQFALGRKFLLQVGVKAKPKLKRAAPTSTRTSSAKRKKVKK

SEQ ID NO: 25 - protein, 504 aa, Artificial
  The sequence is artificially synthesized.
MSVWRPSEATVYLPPVPVSKVVSTDEYVSRTSIYYYAGSSRLLTVGHPYFSIKNTSSGNGKKVLVPKVSGLQYRVFRIKLPDPNKFGFPDTSFYNPETQRLVWACTGLEIGRGQPLGVGISGHPLLNKFDDTETSNKYAGKPGIDNRECLSMDYKQTQLCILGCKPPIGEHWGKGTPCNNNSGNPGDCPPLQLINSVIQDGDMVDTGFGCMDFNTLQASKSDVPIDICSSVCKYPDYLQMASEPYGDSLFFFLRREQMFVRHFFNRAGTLGDPVPGDLYIQGSNSGNTATVQSSAFFPTPSGSMVTSESQLFNKPYWLQRAQGHNNGICWGNQLFVTVVDTTRSTNMTLCAEVKKESTYKNENFKEYLRHGEEFDLQFIFQLCKITLTADVMTYIHKMDATILEDWQFGLTPPPSASLEDTYRFVTSTAITCQKNTPPKGKEDPLKDYMFWEVDLKEKFSADLDQFPLGRKFLLQAGLKAKPKLKRAAPTSTRTSSAKRKKVKK

SEQ ID NO: 26 - protein, 498 aa, Artificial
  The sequence is artificially synthesized.
MATWRPSENKVYLPPTPVSKVVATDSYVKRTSIFYHAGSSRLLAVGHPYYSVTKDNTKTNIPKVSAYQYRVFRVRLPDPNKFGLPDTNIYNPDQERLVWACVGLEVGRGQPLGAGLSGHPLFNRLDDTESSNLANNNVIEDSRDNISVDGKQTQLCIVGCTPAMGEHWTKGAVCKSTQVTTGDCPPLALINTPIEDGDMIDTGFGAMDFKVLQESKAEVPLDIVQSTCKYPDYLKMSADAYGDSMWFYLRREQLFARHYFNRAGKVGETIPAELYLKGSNGREPPPSSVYVATPSGSMITSEAQLFNKPYWLQRAQGHNNGICWGNQLFVTVVDTTRSTNMTISTATEQLSKYDARKINQYLRHVEEYELQFVFQLCKITLSAEVMAYLHNMNANLLEDWNIGLSPPVATSLEDKYRYVRSTAITCQREQPPTEKQDPLAKYKFWDVNLQDSFSTDLDQFPLGRKFLLQAGLKAKPKLKRAAPTSTRTSSAKRKKVKK

SEQ ID NO: 27 - protein, 499 aa, Artificial
  The sequence is artificially synthesized.
MSVWRPSEATVYLPPVPVSKVVSTDEYVSRTSIYYYAGSSRLLAVGNPYFSIKSPNNNKKVLVPKVSGLQYRVFRVRLPDPNKFGFPDTSFYNPDTQRLVWACVGLEIGRGQPLGVGVSGHPYLNKFDDTETSNRYPAQPGSDNRECLSMDYKQTQLCLIGCKPPTGEHWGKGVACNNNAAATDCPPLELFNSIIEDGDMVDTGFGCMDFGTLQANKSDVPIDICNSTCKYPDYLKMASEPYGDSLFFFLRREQMFVRHFFNRAGKLGEAVPDDLYIKGSGNTAVIQSSAFFPTPSGSIVTSESQLFNKPYWLQRAQGHNNGICWGNQLFVTVVDTTRSTNMTLCTEVTKEGTYKNDNFKEYVRHVEEYDLQFVFQLCKITLTAEIMTYIHTMDSNILEDWQFGLTPPPSASLQDTYRFVTSQAITCQKTAPPKEKEDPLNKYTFWEVNLKEKFSADLDQFPLGRKFLLQSGLKAKPKLKRAAPTSTRTSSAKRKKVKK

SEQ ID NO: 28 - protein, 499 aa, Artificial
  The sequence is artificially synthesized.
MSVWRPSEATVYLPPVPVSKVVSTDEYVSRTSIYYYAGSSRLLAVGHPYFSIKNPTNAKKLLVPKVSGLQYRVFRVRLPDPNKFGFPDTSFYNPDTQRLVWACVGLEIGRGQPLGVGISGHPLLNKFDDTETGNKYPGQPGADNRECLSMDYKQTQLCLLGCKPPTGEHWGKGVACTNAAPANDCPPLELINTIIEDGDMVDTGFGCMDFKTLQANKSDVPIDICGSTCKYPDYLKMTSEPYGDSLFFFLRREQMFVRHFFNRAGTLGEAVPDDLYIKGSGTTASIQSSAFFPTPSGSMVTSESQLFNKPYWLQRAQGHNNGICWGNQVFVTVVDTTRSTNMTLCTQVTSDSTYKNENFKEYIRHVEEYDLQFVFQLCKVTLTAEVMTYIHAMNPDILEDWQFGLTPPPSASLQDTYRFVTSQAITCQKTVPPKEKEDPLGKYTFWEVDLKEKFSADLDQFPLGRKFLLQAGLKAKPKLKRAAPTSTRTSSAKRKKVKK

SEQ ID NO: 29 - protein, 508 aa, Artificial
  The sequence is artificially synthesized.
MALWRSSDNKVYLPPPSVAKVVSTDEYVTRTSIFYHAGSSRLLTVGHPYFKVPKGGNGRQDVPKVSAYQYRVFRVKLPDPNKFGLPDNTVYDPNSQRLVWACVGVEIGRGQPLGVGLSGHPLYNKLDDTENSHVASAVDTKDTRDNVSVDYKQTQLCIIGCVPAIGEHWTKGTACKPTTVVQGDCPPLELINTPIEDGDMVDTGYGAMDFKLLQDNKSEVPLDICQSICKYPDYLQMSADAYGDSMFFCLRREQVFARHFWNRSGTMGDQLPESLYIKGTDIRANPGSYLYSPSPSGSVVTSDSQLFNKPYWLHKAQGLNNGICWHNQLFLTVVDTTRSTNLSVCASTTSSIPNVYTPTSFKEYARHVEEFDLQFIFQLCKITLTTEVMSYIHNMNTTILEDWNFGVTPPPTASLVDTYRFVQSAAVTCQKDTAPPVKQDPYDKLKFWPVDLKERFSADLDQFPLGRKFLLQLGARPKPTIGPRKRAAPAPTSTPSPKRVKRRKSSRK

SEQ ID NO: 30 - DNA, 1522 bp, Artificial
  The sequence is artificially synthesized.
ctgggtaccatgtggagaccatctgacagcacagtctatgtgcctcctccaaaccctgtgagcaaggtggtggctacagatgcctatgtgaccaggaccaacatcttctaccatgcctcctccagcagactgctggctgtgggacacccatacttcagcatcaagagggctaacaagacagtggtgccaaaggtgtctggctaccaatacagggtgttcaaggtggtgctgcctgacccaaacaagtttgccctgcctgactcctccctgtttgacccaaccacccagagactggtgtgggcttgtactggattggaggtgggcaggggacaaccactgggagtgggagtgtctggacacccattcctgaacaaatatgatgatgtggagaactctggctctggaggcaaccctggacaagacaacagggtgaatgtggggatggactacaagcagacccaactttgtatggtgggctgtgcccctccactgggagaacactggggcaagggcaagcagtgtaccaacacacctgtccaggctggagactgtcctccattggaactgattacctctgtgattcaggatggagatatggtggacacaggctttggagctatgaactttgctgacctccaaaccaacaagtctgatgtgccaattgacatctgtggcaccacttgtaaataccctgactacctccaaatggctgctgacccatatggagacagactgttcttcttcctgaggaaggaacagatgtttgccagacacttcttcaacagggctggagaggtgggagaacctgtgcctgacaccctgattatcaagggctctggcaacaggacctctgtgggctccagcatctatgtgaacacaccatctggctccctggtgtcctctgaggctcaacttttcaacaagccatactggctccaaaaggctcaaggacacaacaatggcatctgttggggcaaccaactttttgtgacagtggtggacaccaccaggagcaccaatatgaccctgtgtgcctctgtgaccacctccagcacctacaccaactctgactacaaggaatatatgaggcatgtggaggaatatgacctccaattcatcttccaactttgtagcatcaccctgtctgctgaggtgatggcttacatccacacaatgaacccatctgtgttggaggactggaactttggactgagccctcctccaaatggcaccttggaggacacctacagatatgtccagagccaggctatcacttgtcagaagccaacacctgagaaggagaagcctgacccatacaagaacctgtccttctgggaggtgaacctgaaagagaagttctcctctgaactggaccaatacccactgggcaggaagttcctgctccaatctggctacaggggcaggtccagcatcaggacaggagtgaagagacctgctgtgagcaaggcatctgctgccccaaagaggaagagggctaagaccaagaggtaaactcgagctc

SEQ ID NO: 31 - DNA, 1525 bp, Artificial
  The sequence is artificially synthesized.
ctgggtaccatgtggagaccatctgacagcacagtctatgtgcctcctccaaaccctgtgagcaaggtggtggctacagatgcctatgtgaagaggaccaacatcttctaccatgcctcctccagcagactgctggctgtgggacacccatactacagcatcaagaaggtgaacaagacagtggtgccaaaggtgtctggctaccaatacagggtgttcaaggtggtgctgcctgacccaaacaagtttgccctgcctgactcctccctgtttgacccaaccacccagagactggtgtgggcttgtactggattggaggtgggcaggggacaaccactgggagtgggagtgtctggacacccactgctgaacaaatatgatgatgtggagaactctggaggctatggaggcaaccctggacaagacaacagggtgaatgtggggatggactacaagcagacccaactttgtatggtgggctgtgcccctccactgggagaacactggggcaagggcacccagtgtagcaacacctctgtccagaatggagactgtcctccattggaactgattacctctgtgattcaggatggagatatggtggacacaggctttggagctatgaactttgctgacctccaaaccaacaagtctgatgtgccactggacatctgtggcacagtgtgtaaataccctgactacctccaaatggctgctgacccatatggagacagactgttcttctacctgaggaaggaacagatgtttgccagacacttcttcaacagggctggcacagtgggagaacctgtgcctgatgacctgctggtgaagggaggcaacaacaggtcctctgtggcatccagcatctatgtgcatacaccatctggctccctggtgtcctctgaggctcaacttttcaacaagccatactggctccaaaaggctcaaggacacaacaatggcatctgttggggcaaccacctgtttgtgacagtggtggacaccaccaggagcaccaatatgaccctgtgtgcctctgtgagcaagtctgccacctacaccaactctgactacaaggaatatatgaggcatgtggaggagtttgacctccaattcatcttccaactttgtagcatcaccctgtctgctgaggtgatggcttacatccacacaatgaacccatctgtgttggaggactggaactttggactgagccctcctccaaatggcaccttggaggacacctacagatatgtccagagccaggctatcacttgtcagaagccaacacctgagaaggagaagcaggacccatacaaggatatgagtttctgggaggtgaacctgaaagagaagttctcctctgaactggaccagtttccactgggcaggaagttcctgctccaatctggctacaggggcaggacctctgccaggacaggcatcaagagacctgctgtgagcaagccaagcacagccccaaagaggaagaggaccaagaccaagaagtaaactcgagctc

SEQ ID NO: 32 - DNA, 1537 bp, Artificial
  The sequence is artificially synthesized.
ctgggtaccatgagtctgtggctgccatctgaggctacagtctacctgcctcctgtgcctgtgagcaaggtggtgagcacagatgaatatgtggcaaggaccaacatctactaccatgctggcaccagcagactgctggctgtgggacacccatactttccaatcaagaagccaaacaacaacaagattctggtgccaaaggtgtctggactccaatacagggtgttcaggattcacctgcctgacccaaacaagtttggctttcctgacacctccttctacaaccctgacacccagagactggtgtgggcttgtgtgggagtggaggtgggcaggggacaaccactgggagtgggcatctctggacacccactgctgaacaaactggatgacacagagaatgcctctgcctatgctgccaatgctggagtggacaacagggagtgtatcagtatggactacaagcagacccaactttgtctgattggctgtaagcctccaattggagaacactggggcaagggcagcccatgtaccaatgtggctgtgaaccctggagactgtcctccattggaactgataaacacagtgattcaggatggagatatggtggacacaggctttggagctatggacttcaccaccctccaagccaacaagtctgaggtgccactggacatctgtaccagcatctgtaaataccctgactacatcaagatggtgtctgaaccatatggagactccctgttcttctacctgaggagggaacagatgtttgtgagacacctgttcaacagggctggagcagtgggagagaatgtgcctgatgacctctacatcaagggctctggcagcacagccaacctggcatccagcaactactttccaacaccatctggcagtatggtgacctctgatgcccagattttcaacaagccatactggctccaaagggctcaaggacacaacaatggcatctgttggggcaaccaactttttgtgacagtggtggacaccaccaggagcaccaatatgagtctgtgtgctgccatcagcacctctgagaccacctacaagaacaccaacttcaaggaatacctgagacatggagaggaatatgacctccaattcatcttccaactttgtaagattaccctgacagcagatgtgatgacctacatccacagtatgaacagcaccatcttggaggactggaactttggactccaacctcctcctggaggcaccttggaggacacctacaggtttgtgaccagccaggctattgcctgtcagaaacacacacctcctgccccaaaggaggacccactgaaaaaatacaccttctgggaggtgaacctgaaagagaagttctctgctgacctggaccagtttccactgggcaggaagttcctgctccaagcaggactgaaagccaagccaaagttcaccctgggcaagaggaaggctacaccaaccacctccagcaccagcaccacagccaagaggaagaagaggaaactgtaaactcgagctc

SEQ ID NO: 33 - DNA, 1543 bp, Artificial
  The sequence is artificially synthesized.
ctgggtaccatggccctctggagaccatccgataacacagtgtacttgcccccacccagcgtcgcccgggtggtgaacacagacgactacgtcaccagaacctcaatcttctaccacgccgggtccagccggctgctgaccgtgggcaacccctacttccgcgtgcccgccggcggcggaaacaaacaagacatccccaaagtcagcgcctatcagtaccgggtgttccgcgtccaactgcccgatcccaacaagttcggcctgcccgacacctccatctacaaccccgagacccagaggctggtctgggcttgcgccggcgtcgagatcgggaggggccaacccctgggcgtggggttgtccggccaccccttctacaacaagctggacgataccgagtccagccacgcagcaaccagcaacgtctccgaagatgtgcgcgataacgtcagcgtggactacaaacaaacccaactgtgcatcctgggatgcgcacccgccatcggcgagcattgggccaaggggaccgcctgcaagagcaggcccctgagccaaggggactgtccacccctggagttgaagaataccgtgctcgaggacggcgacatggtggacaccggctacggcgctatggatttctccaccctccaggacaccaagtgcgaagtgcccctcgacatctgccaaagcatctgcaagtaccccgactacctccagatgagcgccgacccctacggcgacagcatgttcttctgtctcagaagggaacaattgttcgcccgccacttctggaaccgggccggcacaatgggagatacagtcccccagagcctgtacatcaaggggaccggaatgagggccagccccgggtcctgcgtctacagcccaagcccctccgggagcatcgtcacaagcgatagccaactcttcaacaagccctactggctccacaaagcccaaggccacaataacggggtgtgttggcacaaccagctgttcgtgaccgtcgtggacacaaccaggtccacaaacctgaccatctgcgccagcacccaaagccccgtgcccggccagtacgacgccacaaagttcaaacaatactctcggcacgtggaagagtacgacctccaattcatcttccaactctgcaccatcaccctcaccgccgacgtgatgagctacatccactccatgaactcctccatcctggaagactggaatttcggcgtgccaccaccccctaccacctccctcgtcgacacctacagattcgtgcagagcgtggccatcacatgccagaaagacgccgcccccgccgagaacaaagacccatacgacaaactgaaattctggaacgtcgacctgaaagagaaattcagcctggatctggaccagtacccattgggcaggaagttcctcgtgcaagccggcctcaggagaaaaccaacaatcgggcccaggaagaggagcgcccccagcgcaaccaccagcagcaagcccgcaaaaagggtcagagtgagggcacgcaaataaactcgagctc

SEQ ID NO: 34 - DNA, 1534 bp, Artificial
  The sequence is artificially synthesized.
ctgggtaccatgagcctgtggaggcccagcgaggccaccgtgtacctgccccccgtgcccgtgagcaaggtggtgagcaccgacgagtacgtgaccaggaccaacatctactaccacgccggcagcgccaggctgctgaccgtgggccacccctactacagcatccccaagagcgacaaccccaagaagatcgtggtgcccaaggtgagcggcctgcagtacagggtgttcagggtgaggctgcccgaccccaacaagttcggcttccccgacaccagcttctacaaccccgagacccagaggctggtgtgggcctgcgtgggcctggaggtgggcaggggccagcccctgggcgtgggcatcagcggccaccccctgctgaacaagttcgacgacaccgagaacagcaacaggtacgccggcggccccggcaccgacaacagggagtgcatcagcatggactacaagcagacccagctgtgcctgctgggctgcaagccccccatcggcgagcactggggcaagggcagcccctgcagcaacaacgccatcacccccggcgactgcccccccctggagctgaagaacagcgtgatccaggacggcgacatggtggacaccggcttcggcgccatggacttcaccgccctgcaggacaccaagagcaacgtgcccctggacatctgcaacagcatctgcaagtaccccgactacctgaagatggtggccgagccctacggcgacaccctgttcttctacctgaggagggagcagatgttcgtgaggcacttcttcaacaggagcggcaccgtgggcgagagcgtgcccaccgacctgtacatcaagggcagcggcagcaccgccaccctggccaacagcacctacttccccacccccagcggcagcatggtgaccagcgacgcccagatcttcaacaagccctactggatgcagagggcccagggccacaacaacggcatctgctggggcaaccagctgttcgtgaccgtggtggacaccaccaggagcaccaacatgagcgtgtgcgccgccatcgccaacagcgacaccaccttcaagagcagcaacttcaaggagtacctgaggcacggcgaggagttcgacctgcagttcatcttccagctgtgcaagatcaccctgagcgccgacatcatgacctacatccacagcatgaaccccgccatcctggaggactggaacttcggcctgaccaccccccccagcggcagcctggaggacacctacaggttcgtgaccagccaggccatcacctgccagaagtccgccccccagaagcccaaggaggaccccttcaaggactacgtgttctgggaggtgaacctgaaggagaagttcagcgccgacctggaccagttccccctgggcaggaagttcctgctgcaggccggctacagggccaggcccaagttcaaggccggcaagaggagcgcccccagcgccagcaccaccacccccgccaagaggaagaagaccaagaagtaaactcgagctc

SEQ ID NO: 35 - DNA, 1528 bp, Artificial
  The sequence is artificially synthesized.
ctgggtaccatgagtctgtggaggagcaatgaggctacagtctacctgcctcctgtgtctgtgagcaaggtggtgagcacagatgaatatgtgaccaggaccaacatctactaccatgctggctccagcagactgctggctgtgggacacccatactatgccatcaagaagcaggacagcaacaagattgctgtgccaaaggtgtctggactccaatacagggtgttcagggtgaaactgcctgacccaaacaagtttggctttcctgacacctccttctatgaccctgccagccagagactggtgtgggcttgtactggagtggaggtgggcaggggacaaccactgggagtgggcatctctggacacccactgctgaacaaactggatgacacagagaacagcaacaaatatgtgggcaactctggcacagacaacagggagtgtatcagtatggactacaagcagacccaactttgtctgattggctgtagacctccaattggagaacactggggcaagggcacaccatgtaatgccaaccaggtgaaggctggagagtgtcctccattggaactgctgaacacagtgctccaagatggagatatggtggacacaggctttggagctatggacttcaccaccctccaagccaacaagtctgatgtgccactggacatctgttccagcatctgtaaataccctgactacctgaaaatggtgtctgaaccatatggagatatgctgttcttctacctgaggagggaacagatgtttgtgagacacctgttcaacagggctggcacagtgggagagacagtgcctgctgacctctacatcaagggcaccacaggcaccctgccaagcacctcctactttccaacaccatctggcagtatggtgacctctgatgcccagattttcaacaagccatactggctccaaagggctcaaggacacaacaatggcatctgttggagcaaccaactttttgtgacagtggtggacaccaccaggagcaccaatatgagtgtgtgttctgctgtgtcctcctctgacagcacctacaagaatgacaacttcaaggaatacctgagacatggagaggaatatgacctccaattcatcttccaactttgtaagattaccctgacagcagatgtgatgacctacatccacagtatgaacccaagcatcttggaggactggaactttggactgacacctcctccatctggcaccttggaggacacctacagatatgtgaccagccaggctgtgacttgtcagaagccatctgccccaaagccaaaggatgacccactgaaaaactacaccttctgggaggtggacctgaaagagaagttctctgctgacctggaccagtttccactgggcaggaagttcctgctccaagcaggactgaaagccagaccaaacttcagactgggcaagagggctgcccctgccagcaccagcaagaagtccagcaccaagaggaggaaggtgaagagctaaactcgagctc

SEQ ID NO: 36 - DNA, 1537 bp, Artificial
  The sequence is artificially synthesized.
ctgggtaccatggctatgtggaggtcctctgacagtatggtctacctgcctcctccatctgtggctaaggtggtgaacacagatgactatgtgaccaggacaggcatctactactatgctggctccagcagactgctgacagtgggacacccatacttcaaggtggggatgaatggaggcaggaagcaggacatcccaaaggtgtctgcctaccaatacagggtgttcagggtgaccctgcctgacccaaacaagttcagcatccctgatgcctccctctacaaccctgagacccagagactggtgtgggcttgtgtgggagtggaggtgggcaggggacaaccactgggagtgggcatctctggacacccactctacaacagacaggatgacacagagaacagcccattctccagcaccaccaacaaggacagcagggacaatgtgtctgtggactacaagcagacccaactttgtatcattggctgtgtgcctgccattggagaacactggggcaagggcaaggcttgtaagccaaacaatgtgagcacaggagactgtcctccattggaactggtgaacacaccaattgaggatggagatatgattgacacaggctatggagctatggactttggagccctccaagagaccaagtctgaggtgccactggacatctgtcagagcatctgtaaataccctgactacctccaaatgagtgctgatgtctatggagacagtatgttcttctgtctgaggagggaacaactttttgccagacacttctggaacaggggagggatggtgggagatgccatccctgcccaactctacatcaagggcacagacatcagggctaaccctggctcctctgtctactgtccaagcccatctggcagtatggtgacctctgacagccaacttttcaacaagccatactggctgcacaaggctcaaggacacaacaatggcatctgttggcacaaccaacttttcctgacagtggtggacaccaccaggagcaccaacttcaccctgagcaccagcattgagtccagcatcccaagcacctatgacccaagcaagttcaaggaatacaccaggcatgtggaggaatatgacctccaattcatcttccaactttgtactgtgaccctgaccacagatgtgatgagttacatccacacaatgaactccagcatcctggacaactggaactttgctgtggctcctcctccatctgcctccctggtggacacctacagatacctccaatctgctgccatcacttgtcagaaggatgcccctgcccctgagaagaaggacccatatgatggactgaagttctggaatgtggacctgagggagaagttctccttggaactggaccagtttccactgggcaggaagttcctgctccaagccagggtgaggaggagaccaaccattggaccaaggaagagacctgctgccagcacctcctcctcctctgccaccaaacacaagaggaagagggtgagcaagtaaactcgagctc

SEQ ID NO: 37 - DNA, 1543 bp, Artificial
  The sequence is artificially synthesized.
ctgggtaccatggctctgtggagaccatctgacagcacagtctacctgcctcctccatctgtggcaagggtggtgaacacagatgactatgtgagcaggaccagcatcttctaccatgctggctccagcagactgctgacagtgggcaacccatacttcagggtggtgccaagtggagcaggcaacaagcaggctgtgccaaaggtgtctgcctaccaatacagggtgttcagggtggctctgcctgacccaaacaagtttggactgcctgacagcaccatctacaaccctgagacccagagactggtgtgggcttgtgtggggatggagattggcaggggacaaccactgggcattggactgtctggacacccattctacaacaaactggatgacacagagtctgcccatgctgccacagcagtgattacccaggatgtgagggacaatgtgtctgtggactacaagcagacccaactttgtatcctgggctgtgtgcctgccattggagaacactgggctaagggcaccctgtgtaagcctgcccaactccaacctggagactgtcctccattggaactgaaaaacaccatcattgaggatggagatatggtggacacaggctatggagctatggacttcagcaccctccaagacaccaagtgtgaggtgccactggacatctgtcagagcatctgtaaataccctgactacctccaaatgagtgctgacccatatggagacagtatgttcttctgtctgaggagggaacaactttttgccagacacttctggaacagggctggagtgatgggagacacagtgccaacagacctctacatcaagggcacctctgccaatatgagggagacacctggctcctgtgtctacagcccaagcccatctggcagcatcaccacctctgacagccaacttttcaacaagccatactggctgcacaaggctcaaggacacaacaatggcatctgttggcacaaccaactttttgtgacagtggtggacaccaccaggagcaccaacctgaccctgtgtgccagcacccagaaccctgtgccaaacacctatgacccaaccaagttcaagcactacagcaggcatgtggaggaatatgacctccaattcatcttccaactttgtaccatcaccctgacagcagaggtgatgagttacatccacagtatgaactccagcatcttggagaactggaactttggagtgcctcctcctccaaccacctccctggtggacacctacaggtttgtccagtctgtggctgtgacttgtcagaaggacaccacacctcctgagaagcaggacccatatgacaaactgaagttctggacagtggacctgaaagagaagttctcctctgacctggaccaatacccactgggcaggaagttcctggtccaggctggactgaggaggagaccaaccattggaccaaggaagagacctgctgccagcaccagcacagccagcagacctgccaagagggtgaggattaggagcaagaagtaaa

SEQ ID NO: 38 - DNA, 1534 bp, Artificial
  The sequence is artificially synthesized.
ctgggtaccatggctctgtggaggaccaatgacagcaaggtctacctgcctcctgcccctgtgagcaggattgtgaacacagaggaatacatcaccaggacaggcatctactactatgctggctccagcagactgattaccctgggacacccatactttccaatcccaaagaccagcaccagggctgccatcccaaaggtgtctgccttccaatacagggtgttcagggtccaacttcctgacccaaacaagtttggactgcctgacccaaacctctacaaccctgacacagacagactggtgtggggctgtgtgggagtggaggtgggcaggggacaaccactgggagtgggactgtctggacacccactgttcaacaaatatgatgacacagagaacagcaggattgccaatggcaatgcccaacaggatgtgagggacaacacctctgtggacaacaagcagacccaactttgtatcattggctgtgcccctccaattggagaacactggggcattggcaccacttgtaagaacacacctgtgcctcctggagactgtcctccattggaactggtgtcctctgtgattcaggatggagatatgattgacacaggctttggagctatggactttgctgccctccaagccaccaagtctgatgtgccactggacatcagccagtctgtgtgtaaataccctgactacctgaaaatgagtgctgacacctatggcaacagtatgttcttccacctgaggagggaacagatttttgccagacactactacaacaaactggtgggagtgggagaggacatcccaaatgactactacatcaagggctctggcaatggcagggacccaattgagtcctacatctactctgccacaccatctggcagtatgattacctctgacagccagattttcaacaagccatactggctgcacagggctcaaggacacaacaatggcatctgttggaacaaccaacttttcatcacttgtgtggacaccaccaggagcaccaacctgaccatcagcacagccacagcagcagtgagcccaaccttcacaccaagcaacttcaagcaatacatcagacatggagaggaatatgaactccaattcatcttccaactttgtaagattaccctgaccacagaggtgatggcttacctgcacacaatggacccaaccatcttggaacagtggaactttggactgaccctgcctccatctgcctccttggaggatgcctacaggtttgtgaggaatgctgccacctcctgtcagaaggacacacctccacaggctaagcctgacccactggctaaatacaagttctgggatgtggacctgaaagagaggttctccctggacctggaccagtttgccctgggcaggaagttcctgctccaagtgggagtccagaggaagccaagacctggactgaaaagacctgcctcctctgcctcctcctcctcctcctcctctgccaagaggaagagggtgaagaagtaaactcgagctc

SEQ ID NO: 39 - DNA, 1531 bp, Artificial
  The sequence is artificially synthesized.
ctgggtaccatgagcgtgtggaggcccagcgaggccaccgtgtacctgccccccgtgcccgtgagcaaggtggtgagcaccgacgagtacgtgagcaggaccagcatctactactacgccggcagcagcaggctgctgaccgtgggccacccctacttcagcatcaagaacaccagcagcggcaacggcaagaaggtgctggtgcccaaggtgagcggcctgcagtacagggtgttcaggatcaagctgcccgaccccaacaagttcggcttccccgacaccagcttctacaaccccgagacccagaggctggtgtgggcctgcaccggcctggagatcggcaggggccagcccctgggcgtgggcatcagcggccaccccctgctgaacaagttcgacgacaccgagaccagcaacaagtacgccggcaagcccggcatcgacaacagggagtgcctgagcatggactacaagcagacccagctgtgcatcctgggctgcaagccccccatcggcgagcactggggcaagggcaccccctgcaacaacaacagcggcaaccccggcgactgcccccccctgcagctgatcaacagcgtgatccaggacggcgacatggtggacaccggcttcggctgcatggacttcaacaccctgcaggccagcaagagcgacgtgcccatcgacatctgcagcagcgtgtgcaagtaccccgactacctgcagatggccagcgagccctacggcgacagcctgttcttcttcctgaggagggagcagatgttcgtgaggcacttcttcaacagggccggcaccctgggcgaccccgtgcccggcgacctgtacatccagggcagcaacagcggcaacaccgccaccgtgcagagcagcgccttcttccccacccccagcggcagcatggtgaccagcgagagccagctgttcaacaagccctactggctgcagagggcccagggccacaacaacggcatctgctggggcaaccagctgttcgtgaccgtggtggacaccaccaggagcaccaacatgaccctgtgcgccgaggtgaagaaggagagcacctacaagaacgagaacttcaaggagtacctgaggcacggcgaggagttcgacctgcagttcatcttccagctgtgcaagatcaccctgaccgccgacgtgatgacctacatccacaagatggacgccaccatcctggaggactggcagttcggcctgacccccccccccagcgccagcctggaggacacctacaggttcgtgaccagcaccgccatcacctgccagaagaacaccccccccaagggcaaggaggaccccctgaaggactacatgttctgggaggtggacctgaaggagaagttcagcgccgacctggaccagttccccctgggcaggaagttcctgctgcaggccggcctgcaggccaggcccaagctgaagaggcccgccagcagcgcccccaggaccagcaccaagaagaagaaggtgaagaggtaaactcgagctc

SEQ ID NO: 40 - DNA, 1519 bp, Artificial
  The sequence is artificially synthesized.
ctgggtaccatggctacctggagaccatctgagaacaaggtctacctgcctccaacacctgtgagcaaggtggtggctacagactcctatgtgaagaggaccagcatcttctaccatgctggctccagcagactgctggctgtgggacacccatactactctgtgaccaaggacaacaccaagaccaacatcccaaaggtgtctgcctaccaatacagggtgttcagggtgagactgcctgacccaaacaagtttggactgcctgacaccaacatctacaaccctgaccaggagagactggtgtgggcttgtgtgggattggaggtgggcaggggacaaccactgggagcaggactgtctggacacccactgttcaacagactggatgacacagagtccagcaacctggctaacaacaatgtgattgaggacagcagggacaacatctctgtggatggcaagcagacccaactttgtattgtgggctgtactcctgctatgggagaacactggaccaagggagcagtgtgtaagagcacccaggtgaccacaggagactgtcctccactggctctgataaacacaccaattgaggatggagatatgattgacacaggctttggagctatggacttcaaggtgctccaagagagcaaggctgaggtgccactggacattgtccagagcacttgtaaataccctgactacctgaaaatgagtgctgatgcctatggagacagtatgtggttctacctgaggagggaacaactttttgccagacactacttcaacagggctggcaaggtgggagagaccatccctgctgaactctacctgaaaggcagcaatggcagggaacctcctccatcctctgtctatgtggctacaccatctggcagtatgattacctctgaggctcaacttttcaacaagccatactggctccaaagggctcaaggacacaacaatggcatctgttggggcaaccaactttttgtgacagtggtggacaccaccaggagcaccaatatgaccatcagcacagccacagaacaacttagcaaatatgatgccaggaagataaaccaatacctgaggcatgtggaggaatatgaactccaatttgtgttccaactttgtaagattaccctgtctgctgaggtgatggcttacctgcacaatatgaatgccaacctgttggaggactggaacattggactgagccctcctgtggctacctccttggaggacaaatacagatatgtgaggagcacagccatcacttgtcagagggaacaacctccaacagagaagcaggacccactggctaaatacaagttctgggatgtgaacctccaagactccttcagcacagacctggaccagtttccactgggcaggaagttcctgatgcaacttggcaccaggagcaagcctgctgtggctaccagcaagaagaggtctgccccaaccagcaccagcacacctgccaagaggaagaggaggtaaactcgagctc

SEQ ID NO: 41 - DNA, 1507 bp, Artificial
  The sequence is artificially synthesized.
ctgggtaccatgagcgtgtggaggcccagcgaggccaccgtgtacctgccccccgtgcccgtgagcaaggtggtgagcaccgacgagtacgtgagcaggaccagcatctactactacgccggcagcagcaggctgctggccgtgggcaacccctacttcagcatcaagagccccaacaacaacaagaaggtgctggtgcccaaggtgagcggcctgcagtacagggtgttcagggtgaggctgcccgaccccaacaagttcggcttccccgacaccagcttctacaaccccgacacccagaggctggtgtgggcctgcgtgggcctggagatcggcaggggccagcccctgggcgtgggcgtgagcggccacccctacctgaacaagttcgacgacaccgagaccagcaacaggtaccccgcccagcccggcagcgacaacagggagtgcctgagcatggactacaagcagacccagctgtgcctgatcggctgcaagccccccaccggcgagcactggggcaagggcgtggcctgcaacaacaacgccgccgccaccgactgcccccccctggagctgttcaacagcatcatcgaggacggcgacatggtggacaccggcttcggctgcatggacttcggcaccctgcaggccaacaagagcgacgtgcccatcgacatctgcaacagcacctgcaagtaccccgactacctgaagatggccagcgagccctacggcgacagcctgttcttcttcctgaggagggagcagatgttcgtgaggcacttcttcaacagggccggcaagctgggcgaggccgtgcccgacgacctgtacatcaagggcagcggcaacaccgccgtgatccagagcagcgccttcttccccacccccagcggcagcatcgtgaccagcgagagccagctgttcaacaagccctactggctgcagagggcccagggccacaacaacggcatctgctggggcaaccagctgttcgtgaccgtggtggacaccaccaggagcaccaacatgaccctgtgcaccgaggtgaccaaggagggcacctacaagaacgacaacttcaaggagtacgtgaggcacgtggaggagtacgacctgcagttcgtgttccagctgtgcaagatcaccctgaccgccgagatcatgacctacatccacaccatggacagcaacatcctggaggactggcagttcggcctgacccccccccccagcgccagcctgcaggacacctacaggttcgtgaccagccaggccatcacctgccagaagaccgccccccccaaggagaaggaggaccccctgaacaagtacaccttctgggaggtgaacctgaaggagaagttcagcgccgacctggaccagttccccctgggcaggaagttcctgctgcagagcggcctgaaggccaagcccaggctgaagaggagcgcccccaccaccagggcccccagcaccaagaggaagaaggtgaagaagtaaa